European Patent Specification EP 3 053 592 B1, published April 23, 2025. Title: Vaccine to induce T-cell. Applicant: MIE University KYOTO University. The sequence listing filed with the application follows.

SEQUENCE LISTING (35 sequences)

SEQ ID NO: 1 - protein, 38 aa, Artificial
  MEN(Y6)
SNPARYEFLYYYYYYQYIHSANVLYYYYYYRGPESRLL

SEQ ID NO: 2 - protein, 38 aa, Artificial
  MEN(G6)
SNPARYEFLGGGGGGQYIHSANVLGGGGGGRGPESRLL

SEQ ID NO: 3 - protein, 38 aa, Artificial
  MEN(P6)
SNPARYEFLPPPPPPQYIHSANVLPPPPPPRGPESRLL

SEQ ID NO: 4 - protein, 38 aa, Artificial
  MEN(T6)
SNPARYEFLTTTTTTQYIHSANVLTTTTTTRGPESRLL

SEQ ID NO: 5 - protein, 38 aa, Artificial
  NME(Y6)
RGPESRLLYYYYYYSNPARYEFLYYYYYYQYIHSANVL

SEQ ID NO: 6 - protein, 38 aa, Artificial
  NME(G6)
RGPESRLLGGGGGGSNPARYEFLGGGGGGQYIHSANVL

SEQ ID NO: 7 - protein, 38 aa, Artificial
  NME(P6)
RGPESRLLPPPPPPSNPARYEFLPPPPPPQYIHSANVL

SEQ ID NO: 8 - protein, 38 aa, Artificial
  ENM(Y6)
QYIHSANVLYYYYYYRGPESRLLYYYYYYSNPARYEFL

SEQ ID NO: 9 - protein, 28 aa, Artificial
  MEN(Y1)
SNPARYEFLYQYIHSANVLYRGPESRLL

SEQ ID NO: 10 - protein, 30 aa, Artificial
  MEN(Y2)
SNPARYEFLYYQYIHSANVLYYRGPESRLL

SEQ ID NO: 11 - protein, 32 aa, Artificial
  MEN(Y3)
SNPARYEFLYYYQYIHSANVLYYYRGPESRLL

SEQ ID NO: 12 - protein, 34 aa, Artificial
  MEN(Y4)
SNPARYEFLYYYYQYIHSANVLYYYYRGPESRLL

SEQ ID NO: 13 - protein, 36 aa, Artificial
  MEN(Y5)
SNPARYEFLYYYYYQYIHSANVLYYYYYRGPESRLL

SEQ ID NO: 14 - protein, 42 aa, Artificial
  MEN(Y8)
SNPARYEFLYYYYYYYYQYIHSANVLYYYYYYYYRGPESRLL

SEQ ID NO: 15 - protein, 46 aa, Artificial
  MEN(Y10)
SNPARYEFLYYYYYYYYYYQYIHSANVLYYYYYYYYYYRGPESRLL

SEQ ID NO: 16 - protein, 40 aa, Homo sapience
GARGPESRLLEFYLAMPFATPMEAELARRSLAQDAPPLPV

SEQ ID NO: 17 - protein, 33 aa, Artificial
  ESO1 LP(Y6)
GPESRLLYYYYYYYLAMPFATPMEAELARRSLA

SEQ ID NO: 18 - protein, 39 aa, Artificial
  NMW(A6)
SLLMWITQCAAAAAANYKRCFPVIAAAAAACMTWNQMNL

SEQ ID NO: 19 - protein, 39 aa, Artificial
  NMW(E6)
SLLMWITQCEEEEEENYKRCFPVIEEEEEECMTWNQMNL

SEQ ID NO: 20 - protein, 39 aa, Artificial
  NMW(G6)
SLLMWITQCGGGGGGNYKRCFPVIGGGGGGCMTWNQMNL

SEQ ID NO: 21 - protein, 39 aa, Artificial
  NMW(H6)
SLLMWITQCHHHHHHNYKRCFPVIHHHHHHCMTWNQMNL

SEQ ID NO: 22 - protein, 39 aa, Artificial
  NMW(N6)
SLLMWITQCNNNNNNNYKRCFPVINNNNNNCMTWNQMNL

SEQ ID NO: 23 - protein, 39 aa, Artificial
  NMW(P6)
SLLMWITQCPPPPPPNYKRCFPVIPPPPPPCMTWNQMNL

SEQ ID NO: 24 - protein, 39 aa, Artificial
  NMW(Q6)
SLLMWITQCQQQQQQNYKRCFPVIQQQQQQCMTWNQMNL

SEQ ID NO: 25 - protein, 39 aa, Artificial
  NMW(S6)
SLLMWITQCSSSSSSNYKRCFPVISSSSSSCMTWNQMNL

SEQ ID NO: 26 - protein, 39 aa, Artificial
  NMW(Y6)
SLLMWITQCYYYYYYNYKRCFPVIYYYYYYCMTWNQMNL

SEQ ID NO: 27 - protein, 9 aa, Artificial
  MA p265
SNPARYEFL

SEQ ID NO: 28 - protein, 9 aa, Artificial
  mERK2 9m
QYIHSANVL

SEQ ID NO: 29 - protein, 8 aa, Artificial
  NY p81
RGPESRLL

SEQ ID NO: 30 - protein, 9 aa, Artificial
  NY P157
SLLMWITQC

SEQ ID NO: 31 - DNA, 135 bp, Artificial
  NMW(Y6)
ggatccatgagcctcctgatgtggattacccaatgctattactactattactacaactataagagatgtttccccgtgatctattactactactactattgctatacatggaatcagatgaacctgtgagaattc

SEQ ID NO: 32 - DNA, 135 bp, Artificial
  NMW(T6)
ggatccatgagcctgctcatgtggatcacacaatgcaccactactaccacaaccaactacaagagatgtttccccgtgattaccacaaccacaactacgtgctatacgtggaatcagatgaacctgtgagaattc

SEQ ID NO: 33 - DNA, 135 bp, Artificial
  NMW(G6)
ggatccatgagcttgctcatgtggatcacccaatgtggaggaggtggtggaggcaactacaagcgatgtttccccgtgataggcggtggaggtggagggtgctacacatggaaccagatgaacctgtgagaattc

SEQ ID NO: 34 - DNA, 135 bp, Artificial
  NMW(P6)
ggatccatgagtctgctgatgtggatcactcagtgtcctccaccaccaccacccaactacaagaggtgtttccccgtgattccaccacctcctcctccatgctatacctggaatcagatgaacctgtgagaattc

SEQ ID NO: 35 - protein, 7 aa, Artificial
  NY p82
GPESRLL